European Patent Application EP 4 124 656 A1, published February 1, 2023. Title: PD-L1 microRNAs. Applicant: Martin-Luther-Universitaet Halle-Wittenberg, Medizinische Fakultaet, Institut für Physiologische Chemie. Application not yet assigned. The sequence listing filed with the application follows.

SEQUENCE LISTING (130 sequences)

SEQ ID NO: 1 - RNA, 22 nt, Artificial Sequence
  hsa-mir-26a-5p
uucaaguaauccaggauaggcu

SEQ ID NO: 2 - RNA, 21 nt, Artificial Sequence
  hsa-miR-26b-5p
uucaaguaauucaggauaggu

SEQ ID NO: 3 - RNA, 22 nt, Artificial Sequence
  hsa-miR-29a-3p
uagcaccaucugaaaucgguua

SEQ ID NO: 4 - RNA, 23 nt, Artificial Sequence
  hsa-miR-103b
ucauagcccuguacaaugcugcu

SEQ ID NO: 5 - RNA, 23 nt, Artificial Sequence
  hsa-miR-181b-5p
aacauucauugcugucggugggu

SEQ ID NO: 6 - RNA, 22 nt, Artificial Sequence
  hsa-miR-181b-5p
caaagaauucuccuuuugggcu

SEQ ID NO: 7 - RNA, 24 nt, Artificial Sequence
  hsa-miR-155-5p
uuaaugcuaaucgugauagggguu

SEQ ID NO: 8 - RNA, 23 nt, Artificial Sequence
  hsa-miR-17-5p
caaagugcuuacagugcagguag

SEQ ID NO: 9 - RNA, 22 nt, Artificial Sequence
  hsa-miR-140-5p
cagugguuuuacccuaugguag

SEQ ID NO: 10 - RNA, 23 nt, Artificial Sequence
  hsa-miR-425-5p
aaugacacgaucacucccguuga

SEQ ID NO: 11 - RNA, 22 nt, Artificial Sequence
  hsa-miR-30b-5p
uguaaacauccuacacucagcu

SEQ ID NO: 12 - RNA, 22 nt, Artificial Sequence
  hsa-miR-574-3p
cacgcucaugcacacacccaca

SEQ ID NO: 13 - RNA, 23 nt, Artificial Sequence
  hsa-miR-29b-3p
uagcaccauuugaaaucaguguu

SEQ ID NO: 14 - RNA, 23 nt, Artificial Sequence
  hsa-miR-9-5p
ucuuugguuaucuagcuguauga

SEQ ID NO: 15 - RNA, 22 nt, Artificial Sequence
  hsa-miR-320b
aaaagcuggguugagagggcaa

SEQ ID NO: 16 - RNA, 22 nt, Artificial Sequence
  hsa-miR-25-3p
cauugcacuugucucggucuga

SEQ ID NO: 17 - RNA, 23 nt, Artificial Sequence
  hsa-miR-103a-3p
agcagcauuguacagggcuauga

SEQ ID NO: 18 - RNA, 20 nt, Artificial Sequence
  hsa-miR-320c
aaaagcuggguugagagggu

SEQ ID NO: 19 - RNA, 21 nt, Artificial Sequence
  hsa-miR-629-5p
uggguuuacguugggagaacu

SEQ ID NO: 20 - RNA, 22 nt, Artificial Sequence
  hsa-miR-24-3p
uggcucaguucagcaggaacag

SEQ ID NO: 21 - RNA, 21 nt, Artificial Sequence
  hsa-miR-3074-5p
guuccugcugaacugagccag

SEQ ID NO: 22 - RNA, 22 nt, Artificial Sequence
  hsa-miR-532-3p
ccucccacacccaaggcuugca

SEQ ID NO: 23 - RNA, 23 nt, Artificial Sequence
  hsa-miR-181a-5p
aacauucaacgcugucggugagu

SEQ ID NO: 24 - RNA, 21 nt, Artificial Sequence
  hsa-miR-27b-3p
uucacaguggcuaaguucugc

SEQ ID NO: 25 - RNA, 23 nt, Artificial Sequence
  hsa-miR-30c-5p
uguaaacauccuacacucucagc

SEQ ID NO: 26 - RNA, 21 nt, Artificial Sequence
  hsa-miR-151a-3p
cuagacugaagcuccuugagg

SEQ ID NO: 27 - RNA, 22 nt, Artificial Sequence
  hsa-miR-4521
gcuaaggaaguccugugcucag

SEQ ID NO: 28 - RNA, 22 nt, Artificial Sequence
  hsa-miR-106b-3p
ccgcacuguggguacuugcugc

SEQ ID NO: 29 - RNA, 21 nt, Artificial Sequence
  hsa-miR-23a-3p
aucacauugccagggauuucc

SEQ ID NO: 30 - RNA, 23 nt, Artificial Sequence
  hsa-miR-20a-5p
uaaagugcuuauagugcagguag

SEQ ID NO: 31 - RNA, 23 nt, Artificial Sequence
  hsa-miR-146b-5p
ugagaacugaauuccauaggcug

SEQ ID NO: 32 - RNA, 21 nt, Artificial Sequence
  hsa-miR-3074-5p
guuccugcugaacugagccag

SEQ ID NO: 33 - RNA, 22 nt, Artificial Sequence
  hsa-miR-30e-5p
uguaaacauccuugacuggaag

SEQ ID NO: 34 - RNA, 21 nt, Artificial Sequence
  hsa-miR-222-3p
agcuacaucuggcuacugggu

SEQ ID NO: 35 - RNA, 22 nt, Artificial Sequence
  hsa-miR-340-5p
uuauaaagcaaugagacugauu

SEQ ID NO: 36 - RNA, 22 nt, Artificial Sequence
  hsa-miR-584-5p
uuaugguuugccugggacugag

SEQ ID NO: 37 - RNA, 20 nt, Artificial Sequence
  hsa-miR-550a-3-5p
agugccugagggaguaagag

SEQ ID NO: 38 - RNA, 23 nt, Artificial Sequence
  hsa-miR-550a-5p
agugccugagggaguaagagccc

SEQ ID NO: 39 - RNA, 23 nt, Artificial Sequence
  hsa-miR-454-3p
uagugcaauauugcuuauagggu

SEQ ID NO: 40 - RNA, 22 nt, Artificial Sequence
  hsa-let-7g-5p
ugagguaguaguuuguacaguu

SEQ ID NO: 41 - RNA, 22 nt, Artificial Sequence
  hsa-miR-122-5p
uggagugugacaaugguguuug

SEQ ID NO: 42 - RNA, 22 nt, Artificial Sequence
  hsa-miR-3591-3p
aaacaccauugucacacuccac

SEQ ID NO: 43 - RNA, 21 nt, Artificial Sequence
  hsa-miR-27a-3p
uucacaguggcuaaguuccgc

SEQ ID NO: 44 - RNA, 22 nt, Artificial Sequence
  hsa-miR-185-3p
aggggcuggcuuuccucugguc

SEQ ID NO: 45 - RNA, 21 nt, Artificial Sequence
  hsa-miR-25-5p
aggcggagacuugggcaauug

SEQ ID NO: 46 - RNA, 22 nt, Artificial Sequence
  hsa-let-7e-5p
ugagguaggagguuguauaguu

SEQ ID NO: 47 - RNA, 22 nt, Artificial Sequence
  hsa-miR-211-5p
uucccuuugucauccuucgccu

SEQ ID NO: 48 - RNA, 23 nt, Artificial Sequence
  hsa-miR-221-3p
agcuacauugucugcuggguuuc

SEQ ID NO: 49 - RNA, 22 nt, Artificial Sequence
  hsa-let-7f-5p
ugagguaguagauuguauaguu

SEQ ID NO: 50 - RNA, 21 nt, Artificial Sequence
  hsa-miR-128-3p
ucacagugaaccggucucuuu

SEQ ID NO: 51 - RNA, 23 nt, Artificial Sequence
  hsa-miR-93-5p
caaagugcuguucgugcagguag

SEQ ID NO: 52 - RNA, 22 nt, Artificial Sequence
  hsa-let-7i-5p
ugagguaguaguuugugcuguu

SEQ ID NO: 53 - RNA, 22 nt, Artificial Sequence
  hsa-let-7c-5p
ugagguaguagguuguaugguu

SEQ ID NO: 54 - RNA, 22 nt, Artificial Sequence
  hsa-miR-378a-3p
acuggacuuggagucagaaggc

SEQ ID NO: 55 - RNA, 23 nt, Artificial Sequence
  hsa-miR-105-5p
ucaaaugcucagacuccuguggu

SEQ ID NO: 56 - RNA, 22 nt, Artificial Sequence
  hsa-let-7b-5p
ugagguaguagguugugugguu

SEQ ID NO: 57 - RNA, 22 nt, Artificial Sequence
  hsa-miR-193a-5p
ugggucuuugcgggcgagauga

SEQ ID NO: 58 - RNA, 22 nt, Artificial Sequence
  hsa-miR-451a
aaaccguuaccauuacugaguu

SEQ ID NO: 59 - RNA, 23 nt, Artificial Sequence
  hsa-miR-103a-2-5p
agcuucuuuacagugcugccuug

SEQ ID NO: 60 - RNA, 20 nt, Artificial Sequence
  hsa-miR-550b-3p
ucuuacucccucaggcacug

SEQ ID NO: 61 - DNA, 69 bp, Artificial Sequence
  5 UTR
agttctgcgcagcttcccgaggctccgcaccagccgcgcttctgtccgcctgcagggcattccagaaag

SEQ ID NO: 62 - DNA, 873 bp, Artificial Sequence
  CDS
atgaggatatttgctgtctttatattcatgacctactggcatttgctgaacgcatttactgtcacggttcccaaggacctatatgtggtagagtatggtagcaatatgacaattgaatgcaaattcccagtagaaaaacaattagacctggctgcactaattgtctattgggaaatggaggataagaacattattcaatttgtgcatggagaggaagacctgaaggttcagcatagtagctacagacagagggcccggctgttgaaggaccagctctccctgggaaatgctgcacttcagatcacagatgtgaaattgcaggatgcaggggtgtaccgctgcatgatcagctatggtggtgccgactacaagcgaattactgtgaaagtcaatgccccatacaacaaaatcaaccaaagaattttggttgtggatccagtcacctctgaacatgaactgacatgtcaggctgagggctaccccaaggccgaagtcatctggacaagcagtgaccatcaagtcctgagtggtaagaccaccaccaccaattccaagagagaggagaagcttttcaatgtgaccagcacactgagaatcaacacaacaactaatgagattttctactgcacttttaggagattagatcctgaggaaaaccatacagctgaattggtcatcccagaactacctctggcacatcctccaaatgaaaggactcacttggtaattctgggagccatcttattatgccttggtgtagcactgacattcatcttccgtttaagaaaagggagaatgatggatgtgaaaaaatgtggcatccaagatacaaactcaaagaagcaaagtgatacacatttggaggagacgtaa

SEQ ID NO: 63 - DNA, 1419 bp, Artificial Sequence
  3 UTR-1
tccagcattggaacttctgatcttcaagcagggattctcaacctgtggtttaggggttcatcggggctgagcgtgacaagaggaaggaatgggcccgtgggatgcaggcaatgtgggacttaaaaggcccaagcactgaaaatggaacctggcgaaagcagaggaggagaatgaagaaagatggagtcaaacagggagcctggagggagaccttgatactttcaaatgcctgaggggctcatcgacgcctgtgacagggagaaaggatacttctgaacaaggagcctccaagcaaatcatccattgctcatcctaggaagacgggttgagaatccctaatttgagggtcagttcctgcagaagtgccctttgcctccactcaatcctcaatttgttttctgcatgactgagagtctcagtgttggaacgggacagtatttatgtatgagtttttcctatttattttgagtctgtgaggtcttcttgtcatgtgagtgtggttgtgaatgatttcttttgaagatatattgtagtagatgttacaattttgtcgccaaactaaacttgctgcttaatgatttgctcacatctagtaaaacatggagtatttgtaaggtgcttggtctcctctataactacaagtatacattggaagcataaagatcaaaccgttggttgcataggatgtcacctttatttaacccattaatactctggttgacctaatcttattctcagacctcaagtgtctgtgcagtatctgttccatttaaatatcagctttacaattatgtggtagcctacacacataatctcatttcatcgctgtaaccaccctgttgtgataaccactattattttacccatcgtacagctgaggaagcaaacagattaagtaacttgcccaaaccagtaaatagcagacctcagactgccacccactgtccttttataatacaatttacagctatattttactttaagcaattcttttattcaaaaaccatttattaagtgcccttgcaatatcaatcgctgtgccaggcattgaatctacagatgtgagcaagacaaagtacctgtcctcaaggagctcatagtataatgaggagattaacaagaaaatgtattattacaatttagtccagtgtcatagcataaggatgatgcgaggggaaaacccgagcagtgttgccaagaggaggaaataggccaatgtggtctgggacggttggatatacttaaacatcttaataatcagagtaattttcatttacaaagagaggtcggtacttaaaataaccctgaaaaataacactggaattccttttctagcattatatttattcctgatttgcctttgccatataatctaatgcttgtttatatagtgtctggtattgtttaacagttctgtct

SEQ ID NO: 64 - DNA, 1403 bp, Artificial Sequence
  3  UTR-2
ggtacttaaaataaccctgaaaaataacactggaattccttttctagcattatatttattcctgatttgcctttgccatataatctaatgcttgtttatatagtgtctggtattgtttaacagttctgtcttttctatttaaatgccactaaattttaaattcatacctttccatgattcaaaattcaaaagatcccatgggagatggttggaaaatctccacttcatcctccaagccattcaagtttcctttccagaagcaactgctactgcctttcattcatatgttcttctaaagatagtctacatttggaaatgtatgttaaaagcacgtatttttaaaatttttttcctaaatagtaacacattgtatgtctgctgtgtactttgctatttttatttattttagtgtttcttatatagcagatggaatgaatttgaagttcccagggctgaggatccatgccttctttgtttctaagttatctttcccatagcttttcattatctttcatatgatccagtatatgttaaatatgtcctacatatacatttagacaaccaccatttgttaagtatttgctctaggacagagtttggatttgtttatgtttgctcaaaaggagacccatgggctctccagggtgcactgagtcaatctagtcctaaaaagcaatcttattattaactctgtatgacagaatcatgtctggaacttttgttttctgctttctgtcaagtataaacttcactttgatgctgtacttgcaaaatcacattttctttctggaaattccggcagtgtaccttgactgctagctaccctgtgccagaaaagcctcattcgttgtgcttgaacccttgaatgccaccagctgtcatcactacacagccctcctaagaggcttcctggaggtttcgagattcagatgccctgggagatcccagagtttcctttccctcttggccatattctggtgtcaatgacaaggagtaccttggctttgccacatgtcaaggctgaagaaacagtgtctccaacagagctccttgtgttatctgtttgtacatgtgcatttgtacagtaattggtgtgacagtgttctttgtgtgaattacaggcaagaattgtggctgagcaaggcacatagtctactcagtctattcctaagtcctaactcctccttgtggtgttggatttgtaaggcactttatcccttttgtctcatgtttcatcgtaaatggcataggcagagatgatacctaattctgcatttgattgtcactttttgtacctgcattaatttaataaaatattcttatttattttgttacttggtacaccagcatgtccattttcttgtttattttgtgtttaataaaatgttcagtttaacatccca

SEQ ID NO: 65 - DNA, 22 bp, Artificial Sequence
  primer
gcccgctctttggttatctagc

SEQ ID NO: 66 - DNA, 50 bp, Artificial Sequence
  primer
gtcgtatccagtgcagggtccgaggtattcgcactggatacgactcatac

SEQ ID NO: 67 - DNA, 20 bp, Artificial Sequence
  primer
gccctagcagcacataatgg

SEQ ID NO: 68 - DNA, 50 bp, Artificial Sequence
  primer
gtcgtatccagtgcagggtccgaggtattcgcactggatacgaccacaaa

SEQ ID NO: 69 - DNA, 21 bp, Artificial Sequence
  primer
gcccctagcagcacgtaaata

SEQ ID NO: 70 - DNA, 50 bp, Artificial Sequence
  primer
gtcgtatccagtgcagggtccgaggtattcgcactggatacgaccgccaa

SEQ ID NO: 71 - DNA, 20 bp, Artificial Sequence
  primer
gccccaaagtgcttacagtg

SEQ ID NO: 72 - DNA, 50 bp, Artificial Sequence
  primer
gtcgtatccagtgcagggtccgaggtattcgcactggatacgacctacct

SEQ ID NO: 73 - DNA, 20 bp, Artificial Sequence
  primer
gccccattgcacttgtctcg

SEQ ID NO: 74 - DNA, 50 bp, Artificial Sequence
  primer
gtcgtatccagtgcagggtccgaggtattcgcactggatacgactcagac

SEQ ID NO: 75 - DNA, 50 bp, Artificial Sequence
  primer
gtcgtatccagtgcagggtccgaggtattcgcactggatacgacagccta

SEQ ID NO: 76 - DNA, 20 bp, Artificial Sequence
  primer
gcccttcaagtaatccagga

SEQ ID NO: 77 - DNA, 50 bp, Artificial Sequence
  primer
gtcgtatccagtgcagggtccgaggtattcgcactggatacgacacctat

SEQ ID NO: 78 - DNA, 21 bp, Artificial Sequence
  primer
cacgcattcacagtggctaag

SEQ ID NO: 79 - DNA, 50 bp, Artificial Sequence
  primer
gtcgtatccagtgcagggtccgaggtattcgcactggatacgacgcggaa

SEQ ID NO: 80 - DNA, 20 bp, Artificial Sequence
  primer
gcccttcacagtggctaagt

SEQ ID NO: 81 - DNA, 50 bp, Artificial Sequence
  primer
gtcgtatccagtgcagggtccgaggtattcgcactggatacgacgcagaa

SEQ ID NO: 82 - DNA, 20 bp, Artificial Sequence
  primer
gccctagcaccatctgaaat

SEQ ID NO: 83 - DNA, 50 bp, Artificial Sequence
  primer
gtcgtatccagtgcagggtccgaggtattcgcactggatacgactaaccg

SEQ ID NO: 84 - DNA, 21 bp, Artificial Sequence
  primer
gccctagcaccatttgaaatc

SEQ ID NO: 85 - DNA, 50 bp, Artificial Sequence
  primer
gtcgtatccagtgcagggtccgaggtattcgcactggatacgacaacact

SEQ ID NO: 86 - DNA, 23 bp, Artificial Sequence
  primer
gccccaatcagcaagtatactgc

SEQ ID NO: 87 - DNA, 50 bp, Artificial Sequence
  primer
gtcgtatccagtgcagggtccgaggtattcgcactggatacgacagggca

SEQ ID NO: 88 - DNA, 18 bp, Artificial Sequence
  primer
gccctggcagtgtcttag

SEQ ID NO: 89 - DNA, 50 bp, Artificial Sequence
  primer
gtcgtatccagtgcagggtccgaggtattcgcactggatacgacacaacc

SEQ ID NO: 90 - DNA, 20 bp, Artificial Sequence
  primer
gcccagcagcattgtacagg

SEQ ID NO: 91 - DNA, 50 bp, Artificial Sequence
  primer
gtcgtatccagtgcagggtccgaggtattcgcactggatacgactcatag

SEQ ID NO: 92 - DNA, 20 bp, Artificial Sequence
  primer
gccctcatagccctgtacaa

SEQ ID NO: 93 - DNA, 50 bp, Artificial Sequence
  primer
gtcgtatccagtgcagggtccgaggtattcgcactggatacgacagcagc

SEQ ID NO: 94 - DNA, 21 bp, Artificial Sequence
  primer
cacgcatgagaactgaattcc

SEQ ID NO: 95 - DNA, 50 bp, Artificial Sequence
  primer
gtcgtatccagtgcagggtccgaggtattcgcactggatacgacaaccca

SEQ ID NO: 96 - DNA, 21 bp, Artificial Sequence
  primer
gccctcagtgcactacagaac

SEQ ID NO: 97 - DNA, 50 bp, Artificial Sequence
  primer
gtcgtatccagtgcagggtccgaggtattcgcactggatacgacacaaag

SEQ ID NO: 98 - DNA, 21 bp, Artificial Sequence
  primer
gccctcagtgcatcacagaac

SEQ ID NO: 99 - DNA, 19 bp, Artificial Sequence
  primer
gccctcagtgcatgacaga

SEQ ID NO: 100 - DNA, 50 bp, Artificial Sequence
  primer
gtcgtatccagtgcagggtccgaggtattcgcactggatacgacccaagt

SEQ ID NO: 101 - DNA, 23 bp, Artificial Sequence
  primer
cacgcattaatgctaatcgtgat

SEQ ID NO: 102 - DNA, 49 bp, Artificial Sequence
  primer
tcgtatccagtgcagggtccgaggtattcgcactggatacgacacccct

SEQ ID NO: 103 - DNA, 22 bp, Artificial Sequence
  primer
cacgcaaacattcaacgctgtc

SEQ ID NO: 104 - DNA, 49 bp, Artificial Sequence
  primer
tcgtatccagtgcagggtccgaggtattcgcactggatacgacactcac

SEQ ID NO: 105 - DNA, 20 bp, Artificial Sequence
  primer
gcccaacattcattgctgtc

SEQ ID NO: 106 - DNA, 50 bp, Artificial Sequence
  primer
gtcgtatccagtgcagggtccgaggtattcgcactggatacgacacccac

SEQ ID NO: 107 - DNA, 20 bp, Artificial Sequence
  primer
gccccaaagaattctccttt

SEQ ID NO: 108 - DNA, 50 bp, Artificial Sequence
  primer
gtcgtatccagtgcagggtccgaggtattcgcactggatacgacagccca

SEQ ID NO: 109 - DNA, 20 bp, Artificial Sequence
  primer
gccctaatactgccgggtaa

SEQ ID NO: 110 - DNA, 50 bp, Artificial Sequence
  primer
gtcgtatccagtgcagggtccgaggtattcgcactggatacgactccatc

SEQ ID NO: 111 - DNA, 50 bp, Artificial Sequence
  primer
gtcgtatccagtgcagggtccgaggtattcgcactggatacgactcgccc

SEQ ID NO: 112 - DNA, 20 bp, Artificial Sequence
  primer
gccaaaagctgggttgagag

SEQ ID NO: 113 - DNA, 21 bp, Artificial Sequence
  primer
gaaacgcatcccctagggcat

SEQ ID NO: 114 - DNA, 50 bp, Artificial Sequence
  primer
gtcgtatccagtgcagggtccgaggtattcgcactggatacgacacacca

SEQ ID NO: 115 - DNA, 23 bp, Artificial Sequence
  primer
gcccggttataaagcaatgagac

SEQ ID NO: 116 - DNA, 50 bp, Artificial Sequence
  primer
gtcgtatccagtgcagggtccgaggtattcgcactggatacgacaatcag

SEQ ID NO: 117 - DNA, 21 bp, Artificial Sequence
  primer
cacgcacagcagcaattcatg

SEQ ID NO: 118 - DNA, 49 bp, Artificial Sequence
  primer
tcgtatccagtgcagggtccgaggtattcgcactggatacgacttcaaa

SEQ ID NO: 119 - DNA, 22 bp, Artificial Sequence
  primer
gcgcaatctggaggtaagaagc

SEQ ID NO: 120 - DNA, 50 bp, Artificial Sequence
  primer
gtcgtatccagtgcagggtccgaggtattcgcactggatacgacaaagtg

SEQ ID NO: 121 - DNA, 20 bp, Artificial Sequence
  primer
ccagtgcagggtccgaggta

SEQ ID NO: 122 - DNA, 25 bp, Artificial Sequence
  primer
cggcagcacatatactaaaattgga

SEQ ID NO: 123 - DNA, 25 bp, Artificial Sequence
  primer
aatatggaacgcttcacgaatttgc

SEQ ID NO: 124 - DNA, 23 bp, Artificial Sequence
  primer
cctggatgatgataagcaaatgc

SEQ ID NO: 125 - DNA, 24 bp, Artificial Sequence
  primer
cagttagagctaattaagaccttc

SEQ ID NO: 126 - DNA, 24 bp, Artificial Sequence
  primer
gggtgatgaaaaagaatccttagg

SEQ ID NO: 127 - DNA, 23 bp, Artificial Sequence
  primer
gtgtaactatgacaagtccttgc

SEQ ID NO: 128 - DNA, 22 bp, Artificial Sequence
  primer
gatgtaatgattctgccaaatg

SEQ ID NO: 129 - DNA, 21 bp, Artificial Sequence
  primer
cctcagaatcaaaatggaacg

SEQ ID NO: 130 - DNA, 3633 bp, Homo sapiens
  CD274 molecule (CD274), transcript variant 1, mRNA
agttctgcgcagcttcccgaggctccgcaccagccgcgcttctgtccgcctgcagggcattccagaaagatgaggatatttgctgtctttatattcatgacctactggcatttgctgaacgcatttactgtcacggttcccaaggacctatatgtggtagagtatggtagcaatatgacaattgaatgcaaattcccagtagaaaaacaattagacctggctgcactaattgtctattgggaaatggaggataagaacattattcaatttgtgcatggagaggaagacctgaaggttcagcatagtagctacagacagagggcccggctgttgaaggaccagctctccctgggaaatgctgcacttcagatcacagatgtgaaattgcaggatgcaggggtgtaccgctgcatgatcagctatggtggtgccgactacaagcgaattactgtgaaagtcaatgccccatacaacaaaatcaaccaaagaattttggttgtggatccagtcacctctgaacatgaactgacatgtcaggctgagggctaccccaaggccgaagtcatctggacaagcagtgaccatcaagtcctgagtggtaagaccaccaccaccaattccaagagagaggagaagcttttcaatgtgaccagcacactgagaatcaacacaacaactaatgagattttctactgcacttttaggagattagatcctgaggaaaaccatacagctgaattggtcatcccagaactacctctggcacatcctccaaatgaaaggactcacttggtaattctgggagccatcttattatgccttggtgtagcactgacattcatcttccgtttaagaaaagggagaatgatggatgtgaaaaaatgtggcatccaagatacaaactcaaagaagcaaagtgatacacatttggaggagacgtaatccagcattggaacttctgatcttcaagcagggattctcaacctgtggtttaggggttcatcggggctgagcgtgacaagaggaaggaatgggcccgtgggatgcaggcaatgtgggacttaaaaggcccaagcactgaaaatggaacctggcgaaagcagaggaggagaatgaagaaagatggagtcaaacagggagcctggagggagaccttgatactttcaaatgcctgaggggctcatcgacgcctgtgacagggagaaaggatacttctgaacaaggagcctccaagcaaatcatccattgctcatcctaggaagacgggttgagaatccctaatttgagggtcagttcctgcagaagtgccctttgcctccactcaatcctcaatttgttttctgcatgactgagagtctcagtgttggaacgggacagtatttatgtatgagtttttcctatttattttgagtctgtgaggtcttcttgtcatgtgagtgtggttgtgaatgatttcttttgaagatatattgtagtagatgttacaattttgtcgccaaactaaacttgctgcttaatgatttgctcacatctagtaaaacatggagtatttgtaaggtgcttggtctcctctataactacaagtatacattggaagcataaagatcaaaccgttggttgcataggatgtcacctttatttaacccattaatactctggttgacctaatcttattctcagacctcaagtgtctgtgcagtatctgttccatttaaatatcagctttacaattatgtggtagcctacacacataatctcatttcatcgctgtaaccaccctgttgtgataaccactattattttacccatcgtacagctgaggaagcaaacagattaagtaacttgcccaaaccagtaaatagcagacctcagactgccacccactgtccttttataatacaatttacagctatattttactttaagcaattcttttattcaaaaaccatttattaagtgcccttgcaatatcaatcgctgtgccaggcattgaatctacagatgtgagcaagacaaagtacctgtcctcaaggagctcatagtataatgaggagattaacaagaaaatgtattattacaatttagtccagtgtcatagcataaggatgatgcgaggggaaaacccgagcagtgttgccaagaggaggaaataggccaatgtggtctgggacggttggatatacttaaacatcttaataatcagagtaattttcatttacaaagagaggtcggtacttaaaataaccctgaaaaataacactggaattccttttctagcattatatttattcctgatttgcctttgccatataatctaatgcttgtttatatagtgtctggtattgtttaacagttctgtcttttctatttaaatgccactaaattttaaattcatacctttccatgattcaaaattcaaaagatcccatgggagatggttggaaaatctccacttcatcctccaagccattcaagtttcctttccagaagcaactgctactgcctttcattcatatgttcttctaaagatagtctacatttggaaatgtatgttaaaagcacgtatttttaaaatttttttcctaaatagtaacacattgtatgtctgctgtgtactttgctatttttatttattttagtgtttcttatatagcagatggaatgaatttgaagttcccagggctgaggatccatgccttctttgtttctaagttatctttcccatagcttttcattatctttcatatgatccagtatatgttaaatatgtcctacatatacatttagacaaccaccatttgttaagtatttgctctaggacagagtttggatttgtttatgtttgctcaaaaggagacccatgggctctccagggtgcactgagtcaatctagtcctaaaaagcaatcttattattaactctgtatgacagaatcatgtctggaacttttgttttctgctttctgtcaagtataaacttcactttgatgctgtacttgcaaaatcacattttctttctggaaattccggcagtgtaccttgactgctagctaccctgtgccagaaaagcctcattcgttgtgcttgaacccttgaatgccaccagctgtcatcactacacagccctcctaagaggcttcctggaggtttcgagattcagatgccctgggagatcccagagtttcctttccctcttggccatattctggtgtcaatgacaaggagtaccttggctttgccacatgtcaaggctgaagaaacagtgtctccaacagagctccttgtgttatctgtttgtacatgtgcatttgtacagtaattggtgtgacagtgttctttgtgtgaattacaggcaagaattgtggctgagcaaggcacatagtctactcagtctattcctaagtcctaactcctccttgtggtgttggatttgtaaggcactttatcccttttgtctcatgtttcatcgtaaatggcataggcagagatgatacctaattctgcatttgattgtcactttttgtacctgcattaatttaataaaatattcttatttattttgttacttggtacaccagcatgtccattttcttgtttattttgtgtttaataaaatgttcagtttaacatccca